European Patent Application EP 4 286 849 A1, published December 6, 2023. Title: METHOD FOR QUANTITATIVE MEASUREMENT OF REDUCING SUGARS, AND FLUORESCENT PROBES USED THEREIN. Applicant: WAINVAM-E. The sequence listing filed with the application follows.

SEQUENCE LISTING (1 sequence)

SEQ ID NO: 1 - DNA, 12 bp, Artificial Sequence
  Artificial sequence
agctacagctac